European Patent Specification EP 3 147 356 B1, published March 13, 2024. Title: Method for inducing differentiation of insulin-producing cells. Applicant: NATIONAL UNIVERSITY CORPORATION KUMAMOTO UNIVERSITY. The sequence listing filed with the application follows.

SEQUENCE LISTING (60 sequences)

SEQ ID NO: 1 - DNA, 20 bp, Artificial Sequence
  primer for GAPDH
cgagatccctccaaaatcaa

SEQ ID NO: 2 - DNA, 21 bp, Artificial Sequence
  primer for OCT3/4
gtattcagccaaacgaccatc

SEQ ID NO: 3 - DNA, 21 bp, Artificial Sequence
  primer for CER1
gccgatagatggaatgaaaat

SEQ ID NO: 4 - DNA, 21 bp, Artificial Sequence
  primer for SOX17
gctttcatggtgtgggctaag

SEQ ID NO: 5 - DNA, 22 bp, Artificial Sequence
  primer for FOXA2
ctgagcgagatctaccagtgga

SEQ ID NO: 6 - DNA, 21 bp, Artificial Sequence
  primer for HNF16
atagctccaaccagactcaca

SEQ ID NO: 7 - DNA, 22 bp, Artificial Sequence
  primer for HNF4a
ccaagagatccatggtgttcaa

SEQ ID NO: 8 - DNA, 23 bp, Artificial Sequence
  primer for PDX1
cttggaaaccaacaactattcac

SEQ ID NO: 9 - DNA, 20 bp, Artificial Sequence
  primer for HNF6
aaatcaccatttcccagcag

SEQ ID NO: 10 - DNA, 20 bp, Artificial Sequence
  primer for NKX6.1
ccaagaagaagcaggactcg

SEQ ID NO: 11 - DNA, 23 bp, Artificial Sequence
  primer for SOX9
aaaggcaactcgtacccaaattt

SEQ ID NO: 12 - DNA, 27 bp, Artificial Sequence
  primer for PROX1
aaagcaaagctcatgtttttttatacc

SEQ ID NO: 13 - DNA, 20 bp, Artificial Sequence
  primer for HLXB9
gcaccagttcaagctcaaca

SEQ ID NO: 14 - DNA, 20 bp, Artificial Sequence
  primer for CDX2
ctcctccccagctcttctct

SEQ ID NO: 15 - DNA, 20 bp, Artificial Sequence
  primer for AFP
tgccaactcagtgaggacaa

SEQ ID NO: 16 - DNA, 20 bp, Artificial Sequence
  primer for NGN3
tcgagagagagcgtgacaga

SEQ ID NO: 17 - DNA, 20 bp, Artificial Sequence
  primer for PAX4
cagactgtggctccttcctc

SEQ ID NO: 18 - DNA, 20 bp, Artificial Sequence
  primer for NEUROD1
ctccttcgttcagacgcttt

SEQ ID NO: 19 - DNA, 20 bp, Artificial Sequence
  primer for INS
catcagaagaggccatcaag

SEQ ID NO: 20 - DNA, 20 bp, Artificial Sequence
  primer for GCG
cagaagaggtcgccattgtt

SEQ ID NO: 21 - DNA, 20 bp, Artificial Sequence
  primer for SST
ccaaccagacggagaatgat

SEQ ID NO: 22 - DNA, 20 bp, Artificial Sequence
  primer for PPY
tgcccatttactctggactc

SEQ ID NO: 23 - DNA, 20 bp, Artificial Sequence
  primer for AMY
attcgcaagtggaatggaga

SEQ ID NO: 24 - DNA, 22 bp, Artificial Sequence
  primer for ISL1
atttccctatgtgttggttgcg

SEQ ID NO: 25 - DNA, 20 bp, Artificial Sequence
  primer for MAF-A
ttcagcaaggaggaggtcat

SEQ ID NO: 26 - DNA, 20 bp, Artificial Sequence
  primer for GCK
ggagagaaagcgctgaggac

SEQ ID NO: 27 - DNA, 20 bp, Artificial Sequence
  primer for UCN3
gagggaagtccactctcggg

SEQ ID NO: 28 - DNA, 20 bp, Artificial Sequence
  primer for IAPP
aggcagatcacaaggtcagg

SEQ ID NO: 29 - DNA, 20 bp, Artificial Sequence
  primer for SLC30A8
tgtcccagagagagaccaga

SEQ ID NO: 30 - DNA, 20 bp, Artificial Sequence
  primer for GLUT1
gattcccaagtgtgagtcgc

SEQ ID NO: 31 - DNA, 23 bp, Artificial Sequence
  primer for GAPDH
catgagtccttccacgataccaa

SEQ ID NO: 32 - DNA, 20 bp, Artificial Sequence
  primer for OCT3/4
ctggttcgctttctctttcg

SEQ ID NO: 33 - DNA, 20 bp, Artificial Sequence
  primer for CER1
aaaatgaacagacccgcatt

SEQ ID NO: 34 - DNA, 18 bp, Artificial Sequence
  primer for SOX17
cagcgccttccacgactt

SEQ ID NO: 35 - DNA, 22 bp, Artificial Sequence
  primer for FOXA2
cagtcgttgaaggagagcgagt

SEQ ID NO: 36 - DNA, 20 bp, Artificial Sequence
  primer for HNF16
aggctgtggatattcgtcaa

SEQ ID NO: 37 - DNA, 22 bp, Artificial Sequence
  primer for HNF4a
ttgatgtagtcctccaagctca

SEQ ID NO: 38 - DNA, 21 bp, Artificial Sequence
  primer for PDX1
attaagcatttcccacaaaca

SEQ ID NO: 39 - DNA, 20 bp, Artificial Sequence
  primer for HNF6
agcttttccaccgaggtttt

SEQ ID NO: 40 - DNA, 20 bp, Artificial Sequence
  primer for NKX6.1
tcaacagctgcgtgattttc

SEQ ID NO: 41 - DNA, 20 bp, Artificial Sequence
  primer for SOX9
agtgggtaatgcgcttggat

SEQ ID NO: 42 - DNA, 26 bp, Artificial Sequence
  primer for PROX1
gtaaaactcacggaaattgctaaacc

SEQ ID NO: 43 - DNA, 24 bp, Artificial Sequence
  primer for HLXB9
gcctttttgctgcgtttccatttc

SEQ ID NO: 44 - DNA, 20 bp, Artificial Sequence
  primer for CDX2
tcttagctgcctttggcttc

SEQ ID NO: 45 - DNA, 20 bp, Artificial Sequence
  primer for AFP
tccaacaggcctgagaaatc

SEQ ID NO: 46 - DNA, 20 bp, Artificial Sequence
  primer for NGN3
ctaccggcgcaaaagaatag

SEQ ID NO: 47 - DNA, 20 bp, Artificial Sequence
  primer for PAX4
gggtgctcatagggaaaaca

SEQ ID NO: 48 - DNA, 20 bp, Artificial Sequence
  primer for NEUROD1
gtggaagacatgggagctgt

SEQ ID NO: 49 - DNA, 21 bp, Artificial Sequence
  primer for INS
tcttgggtgtgtagaagaagc

SEQ ID NO: 50 - DNA, 20 bp, Artificial Sequence
  primer for GCG
tggctagcaggtgatgttgt

SEQ ID NO: 51 - DNA, 20 bp, Artificial Sequence
  primer for SST
agggaagagagatggggtgt

SEQ ID NO: 52 - DNA, 20 bp, Artificial Sequence
  primer for PPY
atctgctctggtgtggcatt

SEQ ID NO: 53 - DNA, 20 bp, Artificial Sequence
  primer for AMY
gcccaacccaatcattaaca

SEQ ID NO: 54 - DNA, 20 bp, Artificial Sequence
  primer for ISL1
cgttcttgctgaagccgatg

SEQ ID NO: 55 - DNA, 20 bp, Artificial Sequence
  primer for MAF-A
cgccagcttctcgtatttct

SEQ ID NO: 56 - DNA, 20 bp, Artificial Sequence
  primer for GCK
ctggtttggggtttgaggtt

SEQ ID NO: 57 - DNA, 21 bp, Artificial Sequence
  primer for UCN3
tgttgaggcagctgaagatgg

SEQ ID NO: 58 - DNA, 19 bp, Artificial Sequence
  primer for IAPP
gtgcaatctcggctcactg

SEQ ID NO: 59 - DNA, 20 bp, Artificial Sequence
  primer for SLC30A8
ccacgacctctgcaatcatg

SEQ ID NO: 60 - DNA, 20 bp, Artificial Sequence
  primer for GLUT1
gacatcattgctggctggag